European Patent Application EP 4 431 521 A1, published September 18, 2024. Title: ANTIBODY-DRUG CONJUGATE AND USE THEREOF. Applicant: SHANGHAI INSTITUTE OF BIOLOGICAL PRODUCTS CO., LTD. Application WO PCT/CN2022/135216, filed November 30, 2022. The sequence listing filed with the application follows.

SEQUENCE LISTING (52 sequences)

SEQ ID NO: 1 - protein, 10 aa, synthetic construct
  REGION 1..10: note = anti-HER3 HCDR1
GYTFSNYWID

SEQ ID NO: 2 - protein, 17 aa, synthetic construct
  REGION 1..17: note = anti-HER3 HCDR2
EILPGSGGTDYNEKFKG

SEQ ID NO: 3 - protein, 8 aa, synthetic construct
  REGION 1..8: note = anti-HER3 HCDR3
DDYDVFAY

SEQ ID NO: 4 - protein, 16 aa, synthetic construct
  REGION 1..16: note = anti-HER3 LCDR1
RSSKSLLHSNGITYLY

SEQ ID NO: 5 - protein, 7 aa, synthetic construct
  REGION 1..7: note = anti-HER3 LCDR2
QMSNLAS

SEQ ID NO: 6 - protein, 9 aa, synthetic construct
  REGION 1..9: note = anti-HER3 LCDR3
AQNLELPWT

SEQ ID NO: 7 - protein, 25 aa, synthetic construct [sequence omitted]

SEQ ID NO: 8 - protein, 14 aa, synthetic construct
  REGION 1..14: note = anti-HER3 HFR2
WVRQAPGQGLEWMG

SEQ ID NO: 9 - protein, 32 aa, synthetic construct
  REGION 1..32: note = anti-HER3 HFR3
KATITADTSTSTAYMELSSLRSEDTAVYYCAR

SEQ ID NO: 10 - protein, 11 aa, synthetic construct
  REGION 1..11: note = anti-HER3 HFR4; anti-Claudin18.2 HFR4
WGQGTLVTVSS

SEQ ID NO: 11 - protein, 23 aa, synthetic construct
  REGION 1..23: note = anti-HER3 LFR1
DIVMTQSPGTLSLSPGERATLSC

SEQ ID NO: 12 - protein, 15 aa, synthetic construct
  REGION 1..15: note = anti-HER3 LFR2
WYQQKPGQAPRLLIY

SEQ ID NO: 13 - protein, 32 aa, synthetic construct
  REGION 1..32: note = anti-HER3 LFR3
GVPDRFSSSGSGTDFTLTISRLEPEDFAVYYC

SEQ ID NO: 14 - protein, 11 aa, synthetic construct
  REGION 1..11: note = anti-HER3 LFR4
FGQGTKVEIKR

SEQ ID NO: 15 - protein, 117 aa, synthetic construct
  REGION 1..117: note = anti-HER3 VH
QVQLVQSGAEVKKPGSSVKVSCKASGYTFSNYWIDWVRQAPGQGLEWMGEILPGSGGTDYNEKFKGKATITADTSTSTAYMELSSLRSEDTAVYYCARDDYDVFAYWGQGTLVTVSS

SEQ ID NO: 16 - protein, 113 aa, synthetic construct
  REGION 1..113: note = anti-HER3 VL
DIVMTQSPGTLSLSPGERATLSCRSSKSLLHSNGITYLYWYQQKPGQAPRLLIYQMSNLASGVPDRFSSSGSGTDFTLTISRLEPEDFAVYYCAQNLELPWTFGQGTKVEIKR

SEQ ID NO: 17 - protein, 447 aa, synthetic construct
  REGION 1..447: note = anti-HER3 HC
QVQLVQSGAEVKKPGSSVKVSCKASGYTFSNYWIDWVRQAPGQGLEWMGEILPGSGGTDYNEKFKGKATITADTSTSTAYMELSSLRSEDTAVYYCARDDYDVFAYWGQGTLVTVSSASTKGPSVFPLAPSSKSTSGGTAALGCLVKDYFPEPVTVSWNSGALTSGVHTFPAVLQSSGLYSLSSVVTVPSSSLGTQTYICNVNHKPSNTKVDKKVEPKSCDKTHTCPPCPAPELLGGPSVFLFPPKPKDTLMISRTPEVTCVVVDVSHEDPEVKFNWYVDGVEVHNAKTKPREEQYNSTYRVVSVLTVLHQDWLNGKEYKCKVSNKALPAPIEKTISKAKGQPREPQVYTLPPSRDELTKNQVSLTCLVKGFYPSDIAVEWESNGQPENNYKTTPPVLDSDGSFFLYSKLTVDKSRWQQGNVFSCSVMHEALHNHYTQKSLSLSPGK

SEQ ID NO: 18 - protein, 219 aa, synthetic construct
  REGION 1..219: note = anti-HER3 LC
DIVMTQSPGTLSLSPGERATLSCRSSKSLLHSNGITYLYWYQQKPGQAPRLLIYQMSNLASGVPDRFSSSGSGTDFTLTISRLEPEDFAVYYCAQNLELPWTFGQGTKVEIKRTVAAPSVFIFPPSDEQLKSGTASVVCLLNNFYPREAKVQWKVDNALQSGNSQESVTEQDSKDSTYSLSSTLTLSKADYEKHKVYACEVTHQGLSSPVTKSFNRGEC

SEQ ID NO: 19 - protein, 11 aa, synthetic construct
  REGION 1..11: note = anti-Claudin18.2 HCDR1
GYSITSGYSWH

SEQ ID NO: 20 - protein, 16 aa, synthetic construct
  REGION 1..16: note = anti-Claudin18.2 HCDR2
YIHYSDNTNYAPSLKS

SEQ ID NO: 21 - protein, 9 aa, synthetic construct
  REGION 1..9: note = anti-Claudin18.2 HCDR3
IYYGNSFVY

SEQ ID NO: 22 - protein, 17 aa, synthetic construct
  REGION 1..17: note = anti-Claudin18.2 LCDR1
KSSQSLLNSGNQKNYLT

SEQ ID NO: 23 - protein, 7 aa, synthetic construct
  REGION 1..7: note = anti-Claudin18.2 LCDR2
WASTRES

SEQ ID NO: 24 - protein, 9 aa, synthetic construct
  REGION 1..9: note = anti-Claudin18.2 LCDR3
QNDYFYPYT

SEQ ID NO: 25 - protein, 25 aa, synthetic construct
  REGION 1..25: note = anti-Claudin18.2 HFR1
QVQLQESGPGLVKPSETLSLTCTVS

SEQ ID NO: 26 - protein, 14 aa, synthetic construct
  REGION 1..14: note = anti-Claudin18.2 HFR2
WIRQPPGKGLEWMG

SEQ ID NO: 27 - protein, 32 aa, synthetic construct
  REGION 1..32: note = anti-Claudin18.2 HFR3
RITISRDTSKNQFSLKLSSVTAADTAVYYCAR

SEQ ID NO: 28 - protein, 23 aa, synthetic construct
  REGION 1..23: note = anti-Claudin18.2 LFR1
DIVMTQSPDSLAVSLGERATINC

SEQ ID NO: 29 - protein, 15 aa, synthetic construct
  REGION 1..15: note = anti-Claudin18.2 LFR2
WYQQKPGQPPKLLIY

SEQ ID NO: 30 - protein, 32 aa, synthetic construct
  REGION 1..32: note = anti-Claudin18.2 LFR3
GVPDRFSGSGSGTDFTLTISSLQAEDVAVYYC

SEQ ID NO: 31 - protein, 11 aa, synthetic construct
  REGION 1..11: note = anti-Claudin18.2 LFR4; anti-FR LFR4
FGGGTKLEIKR

SEQ ID NO: 32 - protein, 118 aa, synthetic construct
  REGION 1..118: note = anti-Claudin18.2 VH
QVQLQESGPGLVKPSETLSLTCTVSGYSITSGYSWHWIRQPPGKGLEWMGYIHYSDNTNYAPSLKSRITISRDTSKNQFSLKLSSVTAADTAVYYCARIYYGNSFVYWGQGTLVTVSS

SEQ ID NO: 33 - protein, 114 aa, synthetic construct
  REGION 1..114: note = anti-Claudin18.2 VL
DIVMTQSPDSLAVSLGERATINCKSSQSLLNSGNQKNYLTWYQQKPGQPPKLLIYWASTRESGVPDRFSGSGSGTDFTLTISSLQAEDVAVYYCQNDYFYPYTFGGGTKLEIKR

SEQ ID NO: 34 - protein, 448 aa, synthetic construct
  REGION 1..448: note = anti-Claudin18.2 HC
QVQLQESGPGLVKPSETLSLTCTVSGYSITSGYSWHWIRQPPGKGLEWMGYIHYSDNTNYAPSLKSRITISRDTSKNQFSLKLSSVTAADTAVYYCARIYYGNSFVYWGQGTLVTVSSASTKGPSVFPLAPSSKSTSGGTAALGCLVKDYFPEPVTVSWNSGALTSGVHTFPAVLQSSGLYSLSSVVTVPSSSLGTQTYICNVNHKPSNTKVDKKVEPKSCDKTHTCPPCPAPELLGGPSVFLFPPKPKDTLMISRTPEVTCVVVDVSHEDPEVKFNWYVDGVEVHNAKTKPREEQYNSTYRVVSVLTVLHQDWLNGKEYKCKVSNKALPAPIEKTISKAKGQPREPQVYTLPPSRDELTKNQVSLTCLVKGFYPSDIAVEWESNGQPENNYKTTPPVLDSDGSFFLYSKLTVDKSRWQQGNVFSCSVMHEALHNHYTQKSLSLSPGK

SEQ ID NO: 35 - protein, 220 aa, synthetic construct
  REGION 1..220: note = anti-Claudin18.2 LC
DIVMTQSPDSLAVSLGERATINCKSSQSLLNSGNQKNYLTWYQQKPGQPPKLLIYWASTRESGVPDRFSGSGSGTDFTLTISSLQAEDVAVYYCQNDYFYPYTFGGGTKLEIKRTVAAPSVFIFPPSDEQLKSGTASVVCLLNNFYPREAKVQWKVDNALQSGNSQESVTEQDSKDSTYSLSSTLTLSKADYEKHKVYACEVTHQGLSSPVTKSFNRGEC

SEQ ID NO: 36 - protein, 10 aa, synthetic construct
  REGION 1..10: note = anti-FR HCDR1
GYTFTGYFMN

SEQ ID NO: 37 - protein, 17 aa, synthetic construct
  REGION 1..17: note = anti-FR HCDR2
RIHPYDGDTFYNQKFQG

SEQ ID NO: 38 - protein, 9 aa, synthetic construct
  REGION 1..9: note = anti-FR HCDR3
YDGSRAMDY

SEQ ID NO: 39 - protein, 15 aa, synthetic construct
  REGION 1..15: note = anti-FR LCDR1
KASQSVSFAGTSLMH

SEQ ID NO: 40 - protein, 7 aa, synthetic construct
  REGION 1..7: note = anti-FR LCDR2
RASNLEA

SEQ ID NO: 41 - protein, 9 aa, synthetic construct
  REGION 1..9: note = anti-FR LCDR3
QQSREYPYT

SEQ ID NO: 42 - protein, 25 aa, synthetic construct
  REGION 1..25: note = anti-FR HFR1
QVQLVQSGAEVVKPGASVKISCKAS

SEQ ID NO: 43 - protein, 14 aa, synthetic construct
  REGION 1..14: note = anti-FR HFR2
WVKQSPGQSLEWIG

SEQ ID NO: 44 - protein, 32 aa, synthetic construct
  REGION 1..32: note = anti-FR HFR3
KATLTVDKSSNTAHMELLSLTSEDFAVYYCTR

SEQ ID NO: 45 - protein, 11 aa, synthetic construct
  REGION 1..11: note = anti-FR HFR4
WGQGTTVTVSS

SEQ ID NO: 46 - protein, 23 aa, synthetic construct
  REGION 1..23: note = anti-FR LFR1
DIVLTQSPLSLAVSLGQPAIISC

SEQ ID NO: 47 - protein, 15 aa, synthetic construct
  REGION 1..15: note = anti-FR LFR2
WYHQKPGQQPRLLIY

SEQ ID NO: 48 - protein, 32 aa, synthetic construct
  REGION 1..32: note = anti-FR LFR3
GVPDRFSGSGSKTDFTLTISPVEAEDAATYYC

SEQ ID NO: 49 - protein, 118 aa, synthetic construct
  REGION 1..118: note = anti-FR VH
QVQLVQSGAEVVKPGASVKISCKASGYTFTGYFMNWVKQSPGQSLEWIGRIHPYDGDTFYNQKFQGKATLTVDKSSNTAHMELLSLTSEDFAVYYCTRYDGSRAMDYWGQGTTVTVSS

SEQ ID NO: 50 - protein, 112 aa, synthetic construct
  REGION 1..112: note = anti-FR VL
DIVLTQSPLSLAVSLGQPAIISCKASQSVSFAGTSLMHWYHQKPGQQPRLLIYRASNLEAGVPDRFSGSGSKTDFTLTISPVEAEDAATYYCQQSREYPYTFGGGTKLEIKR

SEQ ID NO: 51 - protein, 448 aa, synthetic construct
  REGION 1..448: note = anti-FR HC
QVQLVQSGAEVVKPGASVKISCKASGYTFTGYFMNWVKQSPGQSLEWIGRIHPYDGDTFYNQKFQGKATLTVDKSSNTAHMELLSLTSEDFAVYYCTRYDGSRAMDYWGQGTTVTVSSASTKGPSVFPLAPSSKSTSGGTAALGCLVKDYFPEPVTVSWNSGALTSGVHTFPAVLQSSGLYSLSSVVTVPSSSLGTQTYICNVNHKPSNTKVDKKVEPKSCDKTHTCPPCPAPELLGGPSVFLFPPKPKDTLMISRTPEVTCVVVDVSHEDPEVKFNWYVDGVEVHNAKTKPREEQYNSTYRVVSVLTVLHQDWLNGKEYKCKVSNKALPAPIEKTISKAKGQPREPQVYTLPPSRDELTKNQVSLTCLVKGFYPSDIAVEWESNGQPENNYKTTPPVLDSDGSFFLYSKLTVDKSRWQQGNVFSCSVMHEALHNHYTQKSLSLSPGK

SEQ ID NO: 52 - protein, 218 aa, synthetic construct
  REGION 1..218: note = anti-FR LC
DIVLTQSPLSLAVSLGQPAIISCKASQSVSFAGTSLMHWYHQKPGQQPRLLIYRASNLEAGVPDRFSGSGSKTDFTLTISPVEAEDAATYYCQQSREYPYTFGGGTKLEIKRTVAAPSVFIFPPSDEQLKSGTASVVCLLNNFYPREAKVQWKVDNALQSGNSQESVTEQDSKDSTYSLSSTLTLSKADYEKHKVYACEVTHQGLSSPVTKSFNRGEC